European Patent Application EP 4 335 456 A1, published March 13, 2024. Title: Binding molecule against dll3 and use thereof. Applicant: SHANGHAI QILU PHARMACEUTICAL RESEARCH AND DEVELOPMENT CENTRE LTD. The sequence listing filed with the application follows.

SEQUENCE LISTING (114 sequences)

SEQ ID NO: 1 - protein, 127 aa, Artificial Sequence
  synthetically generated protein
DVQLVESGGGSVQAGGSLKLSCKSPTYTISSGYMGWFRQAPGKEREGVAAIYIGGSTTLYADSVKGRFTISADNAEKTVYLQMNTLKPEDSAMYYCAAQLRPNSAYHPLDGRKYNYWGQGTQVTVSS

SEQ ID NO: 2 - protein, 116 aa, Artificial Sequence
  synthetically generated protein
QVQLVESGGGLVQPGESLRLSCAGSGFAFSSYDMHWVRQAPGKDFEWVSSISRDGRGPRYADFVKGRFTISKDNGRNMLYLQLNSLEIEDTAMYYCSKGYPIMGGTTQGTQVTVSS

SEQ ID NO: 3 - protein, 118 aa, Artificial Sequence
  synthetically generated protein
QVQLVESGGGSVQAGGSLRLSCAASGDIYSSSYVGWFRQAPGKEREGVAIIYTSGDSTYYANSVKGRFTISQDKAKKTLYLQMNSLKPEDTAMYYCAARFAIDNSNYWGQGTQVTVSS

SEQ ID NO: 4 - protein, 124 aa, Artificial Sequence
  synthetically generated protein
QVQLVESGGGSVQAGGSLRLSCTASGDTYRSYCMGWFRKAPGKEREGVADIVSDGSTSYADSVKGRFTISKDNAKNTLYLQMNSLKPEDTAMYYCAVDRGGSGGYCYTGRYDYWGQGTQVTVSS

SEQ ID NO: 5 - protein, 118 aa, Artificial Sequence
  synthetically generated protein
QVQLVESGGGSVQAGGSLNLSCATSGSTASTTYMGWFRQAPGKGREGVAIIYTARDNPWYANSVKGRFIISQDNAKKTLYLQMNTLKPEDTATYYCAATLANPTRTAWGQGTLVTVSS

SEQ ID NO: 6 - protein, 5 aa, Artificial Sequence
  synthetically generated protein
SGYMG

SEQ ID NO: 7 - protein, 18 aa, Artificial Sequence
  synthetically generated protein
AAIYIGGSTTLYADSVKG

SEQ ID NO: 8 - protein, 18 aa, Artificial Sequence
  synthetically generated protein
QLRPNSAYHPLDGRKYNY

SEQ ID NO: 9 - protein, 5 aa, Artificial Sequence
  synthetically generated protein
SYDMH

SEQ ID NO: 10 - protein, 18 aa, Artificial Sequence
  synthetically generated protein
SSISRDGRGPRYADFVKG

SEQ ID NO: 11 - protein, 7 aa, Artificial Sequence
  synthetically generated protein
GYPIMGG

SEQ ID NO: 12 - protein, 5 aa, Artificial Sequence
  synthetically generated protein
SSYVG

SEQ ID NO: 13 - protein, 18 aa, Artificial Sequence
  synthetically generated protein
AIIYTSGDSTYYANSVKG

SEQ ID NO: 14 - protein, 9 aa, Artificial Sequence
  synthetically generated protein
RFAIDNSNY

SEQ ID NO: 15 - protein, 6 aa, Artificial Sequence
  synthetically generated protein
RSYCMG

SEQ ID NO: 16 - protein, 17 aa, Artificial Sequence
  synthetically generated protein
ADIVSDGSTSYADSVKG

SEQ ID NO: 17 - protein, 16 aa, Artificial Sequence
  synthetically generated protein
DRGGSGGYCYTGRYDY

SEQ ID NO: 18 - protein, 5 aa, Artificial Sequence
  synthetically generated protein
TTYMG

SEQ ID NO: 19 - protein, 17 aa, Artificial Sequence
  synthetically generated protein
IIYTARDNPWYANSVKG

SEQ ID NO: 20 - protein, 9 aa, Artificial Sequence
  synthetically generated protein
TLANPTRTA

SEQ ID NO: 21 - protein, 127 aa, Artificial Sequence
  synthetically generated protein
EVQLVESGGGLVQPGGSLRLSCAASTYTISSGYMGWFRQAPGKEREGVAAIYIGGSTTLYADSVKGRFTISRDNSKNTLYLQMNSLRAEDTAVYYCAAQLRPNSAYHPLDGRKYNYWGQGTLVTVSS

SEQ ID NO: 22 - protein, 127 aa, Artificial Sequence
  synthetically generated protein
EVQLVESGGGLVQPGGSLRLSCKSPTYTISSGYMGWFRQAPGKEREGVAAIYIGGSTTLYADSVKGRFTISRDNSKNTLYLQMNSLRAEDTAVYYCAAQLRPNSAYHPLDGRKYNYWGQGTLVTVSS

SEQ ID NO: 23 - protein, 116 aa, Artificial Sequence
  synthetically generated protein
QVQLVESGGGVVQPGRSLRLSCAASGFAFSSYDMHWVRQAPGKGLEWVSSISRDGRGPRYADSVKGRFTISRDNSKNTLYLQMNSLRAEDTAVYYCSKGYPIMGGTTQGTLVTVSS

SEQ ID NO: 24 - protein, 116 aa, Artificial Sequence
  synthetically generated protein
QVQLVESGGGVVQPGRSLRLSCAASGFAFSSYDMHWVRQAPGKDFEWVSSISRDGRGPRYADSVKGRFTISRDNSKNTLYLQMNSLRAEDTAVYYCSKGYPIMGGTTQGTLVTVSS

SEQ ID NO: 25 - protein, 118 aa, Artificial Sequence
  synthetically generated protein
EVQLVESGGGLVQPGGSLRLSCAASGDIYSSSYVGWFRQAPGKEREGVAIIYTSGDSTYYADSVKGRFTISRDNSKNTLYLQMNSLRAEDTAVYYCAARFAIDNSNYWGQGTLVTVSS

SEQ ID NO: 26 - protein, 124 aa, Artificial Sequence
  synthetically generated protein
EVQLVESGGGLVQPGGSLRLSCAASGDTYRSYCMGWFRQAPGKEREGVADIVSDGSTSYADSVKGRFTISRDNSKNTLYLQMNSLRAEDTAVYYCAVDRGGSGGYCYTGRYDYWGQGTLVTVSS

SEQ ID NO: 27 - protein, 118 aa, Artificial Sequence
  synthetically generated protein
QVQLVESGGGVVQPGGSLRLSCAASGSTASTTYMGWFRQAPGKGREGVAIIYTARDNPWYADSVKGRFTISRDNSKNTLYLQMNSLRAEDTAVYYCAATLANPTRTAWGQGTLVTVSS

SEQ ID NO: 28 - protein, 127 aa, Artificial Sequence
  synthetically generated protein
EVQLVESGGGLVQPGGSLRLSCAASTYTISSGYMGWFRQAPGKEREGVAAIYIGGSTTLYADSVKGRFTISRDNSKNTLYLQMNSLRAEDTAVYYCAAQLRPNAAYHPLDGRKYNYWGQGTLVTVSS

SEQ ID NO: 29 - protein, 127 aa, Artificial Sequence
  synthetically generated protein
EVQLVESGGGLVQPGGSLRLSCAASTYTISSGYMGWFRQAPGKEREGVAAIYIGGSTTLYADSVKGRFTISRDNSKNTLYLQMNSLRAEDTAVYYCAAQLRPQSAYHPLDGRKYNYWGQGTLVTVSS

SEQ ID NO: 30 - protein, 118 aa, Artificial Sequence
  synthetically generated protein
QVQLQQPGAELVKPGASVKLSCKASGYSFTSYWMHWVKQRPGQGLEWIGMIHPTLGDTNYNEKFKSKATLTVDKSSSTAYMELSSLTSEDSAVYYCARLGSLSMMDYWGQGTSVTVSS

SEQ ID NO: 31 - protein, 107 aa, Artificial Sequence
  synthetically generated protein
DIQMTQTTSSLSASLGDRVTISCSASQGISNYLNWYQQKPDGTVKLLIYYTSSLHSGVPARFSGSGSGTDYSLTISNLEPEDIAIYYCQQYSKFPYTFGGGTKLEIK

SEQ ID NO: 32 - protein, 122 aa, Artificial Sequence
  synthetically generated protein
QVQLQQSGAELVKPGASVKMSCKASGYTFISYWITWVKQRPGQGLEWIGDIYPGSGSTTNYNEKFKSKATLTVDTSSSTAYMQLSSLTSEDSAVYYCARETTVGGAYAMDYWGQGTSVTVSS

SEQ ID NO: 33 - protein, 107 aa, Artificial Sequence
  synthetically generated protein
DIVLTQSPATLSVTPGDSVSLSCRASQSINNNLHWYQQKSHESPRLLIKYVSQSISGIPSRFSGSGSGTDFTLTINSVETEDFGMYFCQQTNSWPLTFGAGTKLELK

SEQ ID NO: 34 - protein, 121 aa, Artificial Sequence
  synthetically generated protein
QVQLKQSGPGLVQPSQSLSITCTVSGFSLTSYGVHWVRQSPGKGLEWLGVIWSGGSTDYNAAFISRLSISKDNPKSQVFFKMNSLQADDTAIYYCARENYYGNSLWFFDVWGTGTTVTVSS

SEQ ID NO: 35 - protein, 113 aa, Artificial Sequence
  synthetically generated protein
QVQLQQSGAELVKPGASVKISCKASGYAFSSQWMNWVKQRPGKGLEWIGQIYPGNGDTNYNGKFKGKATLTADKSSSTAYIQLSSLTSEDSAVYFCARWFAYWGQGTLVTVSA

SEQ ID NO: 36 - protein, 107 aa, Artificial Sequence
  synthetically generated protein
DIVLTQSPVTLSVTPGDSVSLSCRASQSVRNNLHWYQQKSHESPRLLIKYVSQSISGIPSRFSGSGSGTDFTLSINSVETEDFGVYFCQQSNSWPLTFGAGTKLELK

SEQ ID NO: 37 - protein, 116 aa, Artificial Sequence
  synthetically generated protein
QVQLQQSDAELVKPGASVKISCKVSGYTFTDHTIHWMKQRPEQGLEWIGYIYPRDGYTMYNEKFKGKATLTADKSSSTAYMQLNSLTSEDSAVHFCARAFHALDYWGQGTSVTVSS

SEQ ID NO: 38 - protein, 107 aa, Artificial Sequence
  synthetically generated protein
DIQMTQTTSSLSASLGDRVTFTCSASQGISNYLNWYQQKPDGTIKLLIYYTSSLHSGVPSRFSGSGSGTDYSLTISNLEPEDIATYYCQQYSKLPYTFGGGTKLEIK

SEQ ID NO: 39 - protein, 116 aa, Artificial Sequence
  synthetically generated protein
EVQLVESGGGLVKPGGSLKLSCAASGFTFSDYGMHWVRQAPEKGLEWVAYISSGSSTIYYADTVKGRFTISRDNAKNTLFLQMTSLRSEDTAMYYCARNSRGFAYWGQGTLVTVSA

SEQ ID NO: 40 - protein, 106 aa, Artificial Sequence
  synthetically generated protein
DIVLTQSPAIMSASPGEKVTMTCSASSSVSYMYWYQQKPGSSPRLLIYDTSNLASGVPVRFSGSGSGTSYSLTISRMEAEDAATYYCQQWSSYPRTFGGGTKLEIK

SEQ ID NO: 41 - protein, 106 aa, Artificial Sequence
  synthetically generated protein
DIVLIQSPTIMSASPGEKVTMTCSASSSVSSMHWYQQKSGTSPKRWIYDTSKLASGVPARFSGSGSGTSYSLTISTMEAEDAATYYCQQWNSYHLTFGAGTKLELK

SEQ ID NO: 42 - protein, 118 aa, Artificial Sequence
  synthetically generated protein
QVQLQQPGAELVKPGTSVKLSCEASGYTFSNYWMQWVRQRPGQGLEWIGMILPNSDITNYNENFQTKATLTVDKSSSTAYMQLSSLTSEDSAVYYCARQARYSAMDYWGQGTSVTVSS

SEQ ID NO: 43 - protein, 107 aa, Artificial Sequence
  synthetically generated protein
DIQMTQTTSSLSVSLGDRVTINCSASQGISNYLNWYQQKPDGTVKLLIYYTSNLHSGVPSRFSGSGSGTDYSLTISNLEPEDIATYYCQHYSKFPYTFGGGTKLEIK

SEQ ID NO: 44 - protein, 121 aa, Artificial Sequence
  synthetically generated protein
QVQLQQPGAELVKPGTSVKLSCKASGYTFTSHWITWVKQRPGQGLEWIGDIYPISGSTNNNEKFRNKATLTVDTSSSTAYMQLSSLTSEDSAVYFCAKIITVGGAYVMDYWGQGTSVTVSS

SEQ ID NO: 45 - protein, 113 aa, Artificial Sequence
  synthetically generated protein
DIVMTQSPSSLAMSVGQKVTMNCKSSQSLLNSSHQKNYLAWYQQKPGQSPKLLVYFASTRESGVPDRFIGSGSGTDFTLTISSVQAEDLADYFCQQHYSTPWTFGGGTKLEIK

SEQ ID NO: 46 - protein, 122 aa, Artificial Sequence
  synthetically generated protein
QVQLVQSGAEVKKPGASVKVSCKASGYTFISYWITWVRQAPGQGLEWMGDIYPGSGSTTNYNEKFKSRVTMTRDTSTSTVYMELSSLRSEDTAVYYCARETTVGGAYAMDYWGQGTLVTVSS

SEQ ID NO: 47 - protein, 107 aa, Artificial Sequence
  synthetically generated protein
EIVLTQSPATLSLSPGERATLSCRASQSINNNLHWYQQKPGQAPRLLIYYVSQSISGIPARFSGSGSGTDFTLTISSLEPEDFAVYYCQQTNSWPLTFGGGTKLEIK

SEQ ID NO: 48 - protein, 107 aa, Artificial Sequence
  synthetically generated protein
EIVLTQSPATLSLSPGERATLSCRASQSINNNLHWYQQKPGQAPRLLIKYVSQSISGIPARFSGSGSGTDFTLTISSLEPEDFAVYYCQQTNSWPLTFGGGTKLEIK

SEQ ID NO: 49 - protein, 116 aa, Artificial Sequence
  synthetically generated protein
QVQLVQSGAEVKKPGASVKVSCKASGYTFTDHTIHWVRQAPGQGLEWMGYIYPRDGYTMYNEKFKGRVTMTRDTSTSTVYMELSSLRSEDTAVYYCARAFHALDYWGQGTLVTVSS

SEQ ID NO: 50 - protein, 107 aa, Artificial Sequence
  synthetically generated protein
DIQMTQSPSSLSASVGDRVTITCSASQGISNYLNWYQQKPGKAPKLLIYYTSSLHSGVPSRFSGSGSGTDFTFTISSLQPEDIATYYCQQYSKLPYTFGGGTKLEIK

SEQ ID NO: 51 - protein, 121 aa, Artificial Sequence
  synthetically generated protein
QVQLVQSGAEVKKPGASVKVSCKASGYTFTSHWITWVRQAPGQGLEWMGDIYPISGSTNNNEKFRNRVTMTRDTSTSTVYMELSSLRSEDTAVYYCAKIITVGGAYVMDYWGQGTLVTVSS

SEQ ID NO: 52 - protein, 107 aa, Artificial Sequence
  synthetically generated protein
EIVMTQSPATLSVSPGERATLSCRASQSVRNNLHWYQQKPGQAPRLLIYYVSQSISGIPARFSGSGSGTEFTLTISSLQSEDFAVYYCQQSNSWPLTFGGGTKLEIK

SEQ ID NO: 53 - protein, 107 aa, Artificial Sequence
  synthetically generated protein
EIVMTQSPATLSVSPGERATLSCRASQSVRNNLHWYQQKPGQAPRLLIKYVSQSISGIPARFSGSGSGTEFTLTISSLQSEDFAVYYCQQSNSWPLTFGGGTKLEIK

SEQ ID NO: 54 - protein, 107 aa, Artificial Sequence
  synthetically generated protein
EIVLTQSPATLSLSPGERATLSCRASQSINNNLHWYQQKPGQAPRLLIKYVSQSISGIPARFSGSGSGTDFTLTISSLEPEDFAVYYCQQTNAWPLTFGGGTKLEIK

SEQ ID NO: 55 - protein, 107 aa, Artificial Sequence
  synthetically generated protein
EIVLTQSPATLSLSPGERATLSCRASQSINNNLHWYQQKPGQAPRLLIKYVSQSISGIPARFSGSGSGTDFTLTISSLEPEDFAVYYCQQTQSWPLTFGGGTKLEIK

SEQ ID NO: 56 - protein, 107 aa, Artificial Sequence
  synthetically generated protein
EIVLTQSPATLSLSPGERATLSCRASQSINNNLHWYQQKPGQAPRLLIKYVSQSISGIPARFSGSGSGTDFTLTISSLEPEDFAVYYCQQTASWPLTFGGGTKLEIK

SEQ ID NO: 57 - protein, 5 aa, Artificial Sequence
  synthetically generated protein
SYWMH

SEQ ID NO: 58 - protein, 17 aa, Artificial Sequence
  synthetically generated protein
MIHPTLGDTNYNEKFKS

SEQ ID NO: 59 - protein, 9 aa, Artificial Sequence
  synthetically generated protein
LGSLSMMDY

SEQ ID NO: 60 - protein, 11 aa, Artificial Sequence
  synthetically generated protein
SASQGISNYLN

SEQ ID NO: 61 - protein, 7 aa, Artificial Sequence
  synthetically generated protein
YTSSLHS

SEQ ID NO: 62 - protein, 9 aa, Artificial Sequence
  synthetically generated protein
QQYSKFPYT

SEQ ID NO: 63 - protein, 5 aa, Artificial Sequence
  synthetically generated protein
SYWIT

SEQ ID NO: 64 - protein, 18 aa, Artificial Sequence
  synthetically generated protein
DIYPGSGSTTNYNEKFKS

SEQ ID NO: 65 - protein, 12 aa, Artificial Sequence
  synthetically generated protein
ETTVGGAYAMDY

SEQ ID NO: 66 - protein, 11 aa, Artificial Sequence
  synthetically generated protein
RASQSINNNLH

SEQ ID NO: 67 - protein, 7 aa, Artificial Sequence
  synthetically generated protein
YVSQSIS

SEQ ID NO: 68 - protein, 9 aa, Artificial Sequence
  synthetically generated protein
QQTNSWPLT

SEQ ID NO: 69 - protein, 5 aa, Artificial Sequence
  synthetically generated protein
SYGVH

SEQ ID NO: 70 - protein, 16 aa, Artificial Sequence
  synthetically generated protein
VIWSGGSTDYNAAFIS

SEQ ID NO: 71 - protein, 13 aa, Artificial Sequence
  synthetically generated protein
ENYYGNSLWFFDV

SEQ ID NO: 72 - protein, 5 aa, Artificial Sequence
  synthetically generated protein
SQWMN

SEQ ID NO: 73 - protein, 17 aa, Artificial Sequence
  synthetically generated protein
QIYPGNGDTNYNGKFKG

SEQ ID NO: 74 - protein, 4 aa, Artificial Sequence
  synthetically generated protein
WFAY

SEQ ID NO: 75 - protein, 11 aa, Artificial Sequence
  synthetically generated protein
RASQSVRNNLH

SEQ ID NO: 76 - protein, 7 aa, Artificial Sequence
  synthetically generated protein
YVSQSIS

SEQ ID NO: 77 - protein, 9 aa, Artificial Sequence
  synthetically generated protein
QQSNSWPLT

SEQ ID NO: 78 - protein, 5 aa, Artificial Sequence
  synthetically generated protein
DHTIH

SEQ ID NO: 79 - protein, 17 aa, Artificial Sequence
  synthetically generated protein
YIYPRDGYTMYNEKFKG

SEQ ID NO: 80 - protein, 7 aa, Artificial Sequence
  synthetically generated protein
AFHALDY

SEQ ID NO: 81 - protein, 11 aa, Artificial Sequence
  synthetically generated protein
SASQGISNYLN

SEQ ID NO: 82 - protein, 7 aa, Artificial Sequence
  synthetically generated protein
YTSSLHS

SEQ ID NO: 83 - protein, 9 aa, Artificial Sequence
  synthetically generated protein
QQYSKLPYT

SEQ ID NO: 84 - protein, 5 aa, Artificial Sequence
  synthetically generated protein
DYGMH

SEQ ID NO: 85 - protein, 17 aa, Artificial Sequence
  synthetically generated protein
YISSGSSTIYYADTVKG

SEQ ID NO: 86 - protein, 7 aa, Artificial Sequence
  synthetically generated protein
NSRGFAY

SEQ ID NO: 87 - protein, 10 aa, Artificial Sequence
  synthetically generated protein
SASSSVSYMY

SEQ ID NO: 88 - protein, 7 aa, Artificial Sequence
  synthetically generated protein
DTSNLAS

SEQ ID NO: 89 - protein, 9 aa, Artificial Sequence
  synthetically generated protein
QQWSSYPRT

SEQ ID NO: 90 - protein, 10 aa, Artificial Sequence
  synthetically generated protein
SASSSVSSMH

SEQ ID NO: 91 - protein, 7 aa, Artificial Sequence
  synthetically generated protein
DTSKLAS

SEQ ID NO: 92 - protein, 9 aa, Artificial Sequence
  synthetically generated protein
QQWNSYHLT

SEQ ID NO: 93 - protein, 5 aa, Artificial Sequence
  synthetically generated protein
NYWMQ

SEQ ID NO: 94 - protein, 17 aa, Artificial Sequence
  synthetically generated protein
MILPNSDITNYNENFQT

SEQ ID NO: 95 - protein, 9 aa, Artificial Sequence
  synthetically generated protein
QARYSAMDY

SEQ ID NO: 96 - protein, 11 aa, Artificial Sequence
  synthetically generated protein
SASQGISNYLN

SEQ ID NO: 97 - protein, 7 aa, Artificial Sequence
  synthetically generated protein
YTSNLHS

SEQ ID NO: 98 - protein, 9 aa, Artificial Sequence
  synthetically generated protein
QHYSKFPYT

SEQ ID NO: 99 - protein, 5 aa, Artificial Sequence
  synthetically generated protein
SHWIT

SEQ ID NO: 100 - protein, 17 aa, Artificial Sequence
  synthetically generated protein
DIYPISGSTNNNEKFRN

SEQ ID NO: 101 - protein, 12 aa, Artificial Sequence
  synthetically generated protein
IITVGGAYVMDY

SEQ ID NO: 102 - protein, 17 aa, Artificial Sequence
  synthetically generated protein
KSSQSLLNSSHQKNYLA

SEQ ID NO: 103 - protein, 7 aa, Artificial Sequence
  synthetically generated protein
FASTRES

SEQ ID NO: 104 - protein, 9 aa, Artificial Sequence
  synthetically generated protein
QQHYSTPWT

SEQ ID NO: 105 - protein, 618 aa, Homo sapiens
  synthetically generated protein
MVSPRMSGLLSQTVILALIFLPQTRPAGVFELQIHSFGPGPGPGAPRSPCSARLPCRLFFRVCLKPGLSEEAAESPCALGAALSARGPVYTEQPGAPAPDLPLPDGLLQVPFRDAWPGTFSFIIETWREELGDQIGGPAWSLLARVAGRRRLAAGGPWARDIQRAGAWELRFSYRARCEPPAVGTACTRLCRPRSAPSRCGPGLRPCAPLEDECEAPLVCRAGCSPEHGFCEQPGECRCLEGWTGPLCTVPVSTSSCLSPRGPSSATTGCLVPGPGPCDGNPCANGGSCSETPRSFECTCPRGFYGLRCEVSGVTCADGPCFNGGLCVGGADPDSAYICHCPPGFQGSNCEKRVDRCSLQPCRNGGLCLDLGHALRCRCRAGFAGPRCEHDLDDCAGRACANGGTCVEGGGAHRCSCALGFGGRDCRERADPCAARPCAHGGRCYAHFSGLVCACAPGYMGARCEFPVHPDGASALPAAPPGLRPGDPQRYLLPPALGLLVAAGVAGAALLLVHVRRRGHSQDAGSRLLAGTPEPSVHALPDALNNLRTQEGSGDGPSSSVDWNRPEDVDPQGIYVISAPSIYAREVATPLFPPLHTGRAGQRQHLLFPYPSSILSVK

SEQ ID NO: 106 - protein, 618 aa, Macaca fascicularis
  synthetically generated protein
MVSPRMSRLLSQTVILALIFIPQARPAGVFELQIHSFGPGPGPGAPRSPCSARGPCRLFFRVCLKPGLSEEAAESPCALGAALSARGPVYTEQPEAPAPDLPLPNGLLQVPFRDAWPGTFSLIIETWREELGDQIGGPAWSLLARVTRRRRLAAGGPWARDIQRAGAWELRFSYRARCELPAVGTACTRLCRPRSAPSRCGPGLRPCAPLEDECEAPPVCRAGCSLEHGFCEQPGECRCLEGWTGPLCMVPVSTSSCLGLRGPSSTTTGCLVPGPGPCDGNPCANGGSCSETPGSFECTCPRGFYGLRCEVSGVTCADGPCFNGGLCVGGADPDSAYICHCPPGFQGSNCEKRVDRCSLQPCRNGGLCLDLGHALRCRCRAGFAGPRCEHDLDDCAGRACANGGTCVEGGGAHRCSCALGFGGRNCRERADPCAARPCAHGGRCYAHFSGLVCACAPGYMGARCEFPVHPDGVSALPAAPPGLRPGDPQRYLLPPALGLLVAAGVAGAALLLVHVRRRGHAQDAGSRLLAGTPEPSVHALPDALNNLRTQEGPGDVPSSSVDWNRPEDVDSRGIYVISAPSIYAREVAMPLFPPLHTGRAGQRQNLLFPFPSSILSVK

SEQ ID NO: 107 - protein, 723 aa, Homo sapiens
  synthetically generated protein
MGSRCALALAVLSALLCQVWSSGVFELKLQEFVNKKGLLGNRNCCRGGAGPPPCACRTFFRVCLKHYQASVSPEPPCTYGSAVTPVLGVDSFSLPDGGGADSAFSNPIRFPFGFTWPGTFSLIIEALHTDSPDDLATENPERLISRLATQRHLTVGEEWSQDLHSSGRTDLKYSYRFVCDEHYYGEGCSVFCRPRDDAFGHFTCGERGEKVCNPGWKGPYCTEPICLPGCDEQHGFCDKPGECKCRVGWQGRYCDECIRYPGCLHGTCQQPWQCNCQEGWGGLFCNQDLNYCTHHKPCKNGATCTNTGQGSYTCSCRPGYTGATCELGIDECDPSPCKNGGSCTDLENSYSCTCPPGFYGKICELSAMTCADGPCFNGGRCSDSPDGGYSCRCPVGYSGFNCEKKIDYCSSSPCSNGAKCVDLGDAYLCRCQAGFSGRHCDDNVDDCASSPCANGGTCRDGVNDFSCTCPPGYTGRNCSAPVSRCEHAPCHNGATCHERGHRYVCECARGYGGPNCQFLLPELPPGPAVVDLTEKLEGQGGPFPWVAVCAGVILVLMLLLGCAAVVVCVRLRLQKHRPPADPCRGETETMNNLANCQREKDISVSIIGATQIKNTNKKADFHGDHSADKNGFKARYPAVDYNLVQDLKGDDTAVRDAHSKRDTKCQPQGSSGEEKGTPTTLRGGEASERKRPDSGCSTSKDTKYQSVYVISEEKDECVIATEV

SEQ ID NO: 108 - protein, 685 aa, Homo sapiens
  synthetically generated protein
MAAASRSASGWALLLLVALWQQRAAGSGVFQLQLQEFINERGVLASGRPCEPGCRTFFRVCLKHFQAVVSPGPCTFGTVSTPVLGTNSFAVRDDSSGGGRNPLQLPFNFTWPGTFSLIIEAWHAPGDDLRPEALPPDALISKIAIQGSLAVGQNWLLDEQTSTLTRLRYSYRVICSDNYYGDNCSRLCKKRNDHFGHYVCQPDGNLSCLPGWTGEYCQQPICLSGCHEQNGYCSKPAECLCRPGWQGRLCNECIPHNGCRHGTCSTPWQCTCDEGWGGLFCDQDLNYCTHHSPCKNGATCSNSGQRSYTCTCRPGYTGVDCELELSECDSNPCRNGGSCKDQEDGYHCLCPPGYYGLHCEHSTLSCADSPCFNGGSCRERNQGANYACECPPNFTGSNCEKKVDRCTSNPCANGGQCLNRGPSRMCRCRPGFTGTYCELHVSDCARNPCAHGGTCHDLENGLMCTCPAGFSGRRCEVRTSIDACASSPCFNRATCYTDLSTDTFVCNCPYGFVGSRCEFPVGLPPSFPWVAVSLGVGLAVLLVLLGMVAVAVRQLRLRRPDDGSREAMNNLSDFQKDNLIPAAQLKNTNQKKELEVDCGLDKSNCGKQQNHTLDYNLAPGPLGRGTMPGKFPHSDKSLGEKAPLRLHSEKPECRISAICSPRDSMYQSVCLISEERNECVIATEV

SEQ ID NO: 109 - protein, 226 aa, Homo sapiens
  synthetically generated protein
DKTHTCPPCPAPELLGGPSVFLFPPKPKDTLMISRTPEVTCVVVDVSHEDPEVKFNWYVDGVEVHNAKTKPREEQYNSTYRVVSVLTVLHQDWLNGKEYKCKVSNKALPAPIEKTISKAKGQPREPQVYTLPPSRDELTKNQVSLTCLVKGFYPSDIAVEWESNGQPENNYKTTPPVLDSDGSFFLYSKLTVDKSRWQQGNVFSCSVMHEALHNHYTQKSLSLSPG

SEQ ID NO: 110 - protein, 18 aa, Artificial Sequence
  synthetically generated protein
QLRPNAAYHPLDGRKYNY

SEQ ID NO: 111 - protein, 18 aa, Artificial Sequence
  synthetically generated protein
QLRPQSAYHPLDGRKYNY

SEQ ID NO: 112 - protein, 9 aa, Artificial Sequence
  synthetically generated protein
QQTNAWPLT

SEQ ID NO: 113 - protein, 9 aa, Artificial Sequence
  synthetically generated protein
QQTQSWPLT

SEQ ID NO: 114 - protein, 9 aa, Artificial Sequence
  synthetically generated protein
QQTASWPLT